European Patent Specification EP 3 374 523 B1, published June 21, 2023. Title: BIOMARKERS FOR PROSPECTIVE DETERMINATION OF RISK FOR DEVELOPMENT OF ACTIVE TUBERCULOSIS. Applicant: University of Cape Town Center for Infectious Disease Research. The sequence listing filed with the application follows.

SEQUENCE LISTING (4 sequences)

SEQ ID NO: 1 - DNA, 568 bp, Homo sapiens
  prim_transcript (1)..(568)
aaccgggtgaacatgacctacgagaagatgtctcgtgccctgcgccactattataagcttaatatcattaagaaggaaccggggcagaaactcctgttcagaaatggacttcagctgatcttcatattcatatggagtttccagtgaccccaaatagccaaaacagtcttggaaagaaaaacaaagttggaggacccacacttcctgattttgaaacttgctacaaagctatagtactcaacaaagattggtaatggcataaggatatagattaagaacagttttttcaacaaatagtgttgggacaatgggtgtccacatgcaaaagaataaagttgtccccttaccttacaccatctccaaaaattaactcaaaatatgtcaaagacataaacgtaagagctaaaactgtaaaactcctagaataaaacataggagtaaatcttcatgaccttggattaggccattgtgtcttaaatataacaccaaaagaataagtaataaaaaaatagataaattgaactccatcaaaattaaaagcctttgtgcttcataggacaccatcaag

SEQ ID NO: 2 - DNA, 446 bp, Homo sapiens
  prim_transcript (1)..(446)
ctatgtgacagagctgacacatagaatccgatcaaaatcctcacctgatgagaatgagaatgaggttgaggattcagctgactttgtgagcttcttcccagactttgtgtggacactgagagatttctccctggacttggaagcagatggacaacccctcacaccagatgagtacctgacatactccctgaagctgaagaaaggtaccagtcaaaaagatgaaacttttaacctgcccagactctgtatccggaaattcttcccaaagaaaaaatgctttgtctttgatcggcccgttcaccgcaggaagcttgcccagctcgagaaactacaagatgaagagctggaccccgaatttgtgcaacaagtagcagacttctgttcctacatctttagtaattccaaaactaaaactctttcaggaggcatccaggtcaacgggcctc

SEQ ID NO: 3 - DNA, 494 bp, Homo sapiens
  prim_transcript (1)..(494)
gtctagagagcctggtgctgacctacgtcaatgccatcagcagtggggatctaccctgcatggagaacgcagtcctggccttggcccagatagagaactcagccgcagtggaaaaggctattgcccactatgaacagcagatgggccagaaggtgcagctgcccacggaaaccctccaggagctgctggacctgcacagggacagtgagagagaggccattgaagtcttcatgaagaactctttcaaggatgtggaccaaatgttccagaggaaattaggggcccagttggaagcaaggcgagatgacttttgtaagcagaattccaaagcatcatcagattgttgcatggctttacttcaggatatatttggccctttagaagaagatgtcaagcagggaacattttctaaaccaggaggttaccgtctctttactcagaagctgcaggagctgaagaataagtactaccaggtgccaaggaaggggatacag

SEQ ID NO: 4 - DNA, 1783 bp, Homo sapiens
  prim_transcript (1)..(1783)
aggcacaagtgaaagcagaagctgaaaaggctgaagcgcaaaggttggcggcgattcaaaggcagaacgagcaaatgatgcaggagagggagagactccatcaggaacaagtgagacaaatggagatagccaaacaaaattggctggcagagcaacagaaaatgcaggaacaacagatgcaggaacaggctgcacagctcagcacaacattccaagctcaaaatagaagccttctcagtgagctccagcacgcccagaggactgttaataacgatgatccatgtgttttactctaaagtgctaaatatgggagtttcctttttttactctttgtcactgatgacacaacagaaaagaaactgtagaccttgggacaatcaacatttaaataaactttataattattttttcaaactttcatatagagttataagattatgatgctggtatctggtaaaatgtacatcccagtagtccaatagtttaaatgtttattgcttcctttaagagattataaattgtataagggacattgtatcactgccttcatttatgcgtgatattgggatggtttcatcaggagatgctttccttgcatctcaatgtcatctgtctaatttctcataaggggattatgttacctagagcagggcttcccaaccctcaggccatagactagctctgatctgtggcctcttaggaacccggccacacagcaggaggtgagcagcaggtaagtgagcattacagcctgagctccacctcctgtcagatcagcagtgacattagattctcacaggagtgggaaccctattgtgaactgtgcatgcaaaagatctaggttgtgtgatccttgtggaacaatataaaccagaaaccaataacgccaccccacctccaacccccgccaaccctctgtggaaaaattaccttccacgaaactggtccctgatgccaaataggttgggggaccgctgacctagagggagttatgcacatgggcttataaggttagccaagagaaaggacaagaagacccaaagtcggcaagcaaatttattaacctgctgggctgctctacagaaatctgaggaggcagacaccgggcttacaggctaaggggtataagtaggtctgcaggggttttgtgtgtgtgtgcgggggtgtcgggggggcaaggccatttgtggagacttttcctcccagtatggccacatcctgcagtttgtcagtttttgcccccgcctggctcagggtaccaggatgtggtttagcttaggggtggttatagtggcacctaagttctgggaacttgcggtgggggcgaccttttggacgaaaaataagctgcagggcagctaggggagggggcttgttatattcctctgggggcagggtgtccctaactgggctcagtcggaaggaacttgaccaaagtctgggctcagttgggcatcactcaggctaatggtcgtgtgctggatgccatcagagggaagtaccaatggtaaagtggaaacaatgtgcagctttcaactgggtggaggctgctattctgtggacagtgagatgtttccttggcactgtcaatagacaatctgcgtagagaaattccaagctgaaagccaataatgttataataaaatagagattcttcagaagatgaaaggaattaccagcatggaaattgtgtcataggcttaagggctaaagaagaagccttttcttttctgttcaccctcaccaagagcacaacttaaatagggcattttataacctgaac